European Patent Application EP 4 807 011 A1, published September 16, 2026. Title: Adeno-associated virus vector capable of astrocyte-specific gene delivery. Applicant: GLUGENETHERAPEUTICS INC. Application KR. The sequence listing filed with the application follows.

SEQUENCE LISTING (11 sequences)

SEQ ID NO: 1 - protein, 736 aa, Adeno-associated virus serotype 1
MAADGYLPDWLEDNLSEGIREWWDLKPGAPKPKANQQKQDDGRGLVLPGYKYLGPFNGLDKGEPVNAADAAALEHDKAYDQQLKAGDNPYLRYNHADAEFQERLQEDTSFGGNLGRAVFQAKKRVLEPLGLVEEGAKTAPGKKRPVEQSPQEPDSSSGIGKTGQQPAKKRLNFGQTGDSESVPDPQPLGEPPATPAAVGPTTMASGGGAPMADNNEGADGVGNASGNWHCDSTWLGDRVITTSTRTWALPTYNNHLYKQISSASTGASNDNHYFGYSTPWGYFDFNRFHCHFSPRDWQRLINNNWGFRPKRLNFKLFNIQVKEVTTNDGVTTIANNLTSTVQVFSDSEYQLPYVLGSAHQGCLPPFPADVFMIPQYGYLTLNNGSQAVGRSSFYCLEYFPSQMLRTGNNFTFSYTFEEVPFHSSYAHSQSLDRLMNPLIDQYLYYLNRTQNQSGSAQNKDLLFSRGSPAGMSVQPKNWLPGPCYRQQRVSKTKTDNNNSNFTWTGASKYNLNGRESIINPGTAMASHKDDEDKFFPMSGVMIFGKESAGASNTALDNVMITDEEEIKATNPVATERFGTVAVNFQSSSTDPATGDVHAMGALPGMVWQDRDVYLQGPIWAKIPHTDGHFHPSPLMGGFGLKNPPPQILIKNTPVPANPPAEFSATKFASFITQYSTGQVSVEIEWELQKENSKRWNPEVQYTSNYAKSANVDFTVDNNGLYTEPRPIGTRYLTRPL

SEQ ID NO: 2 - DNA, 2211 bp, Adeno-associated virus serotype 1
  source 1..2211: mol_type = genomic DNA
atggctgccgatggttatcttccagattggctcgaggacaacctctctgagggcattcgcgagtggtgggacttgaaacctggagccccgaagcccaaagccaaccagcaaaagcaggacgacggccggggtctggtgcttcctggctacaagtacctcggacccttcaacggactcgacaagggggagcccgtcaacgcggcggacgcagcggccctcgagcacgacaaggcctacgaccagcagctcaaagcgggtgacaatccgtacctgcggtataaccacgccgacgccgagtttcaggagcgtctgcaagaagatacgtcttttgggggcaacctcgggcgagcagtcttccaggccaagaagcgggttctcgaacctctcggtctggttgaggaaggcgctaagacggctcctggaaagaaacgtccggtagagcagtcgccacaagagccagactcctcctcgggcatcggcaagacaggccagcagcccgctaaaaagagactcaattttggtcagactggcgactcagagtcagtccccgatccacaacctctcggagaacctccagcaacccccgctgctgtgggacctactacaatggcttcaggcggtggcgcaccaatggcagacaataacgaaggcgccgacggagtgggtaatgcctcaggaaattggcattgcgattccacatggctgggcgacagagtcatcaccaccagcacccgcacctgggccttgcccacctacaataaccacctctacaagcaaatctccagtgcttcaacgggggccagcaacgacaaccactacttcggctacagcaccccctgggggtattttgatttcaacagattccactgccacttttcaccacgtgactggcagcgactcatcaacaacaattggggattccggcccaagagactcaacttcaaactcttcaacatccaagtcaaggaggtcacgacgaatgatggcgtcacaaccatcgctaataaccttaccagcacggttcaagtcttctcggactcggagtaccagcttccgtacgtcctcggctctgcgcaccagggctgcctccctccgttcccggcggacgtgttcatgattccgcaatacggctacctgacgctcaacaatggcagccaagccgtgggacgttcatccttttactgcctggaatatttcccttctcagatgctgagaacgggcaacaactttaccttcagctacacctttgaggaagtgcctttccacagcagctacgcgcacagccagagcctggaccggctgatgaatcctctcatcgaccaatacctgtattacctgaacagaactcaaaatcagtccggaagtgcccaaaacaaggacttgctgtttagccgtgggtctccagctggcatgtctgttcagcccaaaaactggctacctggaccctgttatcggcagcagcgcgtttctaaaacaaaaacagacaacaacaacagcaattttacctggactggtgcttcaaaatataacctcaatgggcgtgaatccatcatcaaccctggcactgctatggcctcacacaaagacgacgaagacaagttctttcccatgagcggtgtcatgatttttggaaaagagagcgccggagcttcaaacactgcattggacaatgtcatgattacagacgaagaggaaattaaagccactaaccctgtggccaccgaaagatttgggaccgtggcagtcaatttccagagcagcagcacagaccctgcgaccggagatgtgcatgctatgggagcattacctggcatggtgtggcaagatagagacgtgtacctgcagggtcccatttgggccaaaattcctcacacagatggacactttcacccgtctcctcttatgggcggctttggactcaagaacccgcctcctcagatcctcatcaaaaacacgcctgttcctgcgaatcctccggcggagttttcagctacaaagtttgcttcattcatcacccaatactccacaggacaagtgagtgtggaaattgaatgggagctgcagaaagaaaacagcaagcgctggaatcccgaagtgcagtacacatccaattatgcaaaatctgccaacgttgattttactgtggacaacaatggactttatactgagcctcgccccattggcacccgttaccttacccgtcccctgtaa

SEQ ID NO: 3 - protein, 736 aa, synthetic construct
MAADGYLPDWLEDNLSEGIREWWDLKPGAPKPKANQQKQDDGRGLVLPGYKYLGPFNGLDKGEPVNAADAAALEHDKAYDQQLKAGDNPYLRYNHADAEFQERLQEDTSFGGNLGRAVFQAKKRVLEPLGLVEEGAKTAPGKKRPVEQSPQEPDSSSGIGKTGQQPAKKRLNFGQTGDSESVPDPQPLGEPPATPAAVGPTTMASGGGAPMADNNEGADGVGNASGNWHCDSTWLGDRVITTSTRTWALPTYNNHLYKQISSASTGASNDNHYFGYSTPWGYFDFNRFHCHFSPRDWQRLINNNWGFRPKRLNFKLFNIQVKEVTTNDGVTTIANNLTSTVQVFSDSEYQLPYVLGSAHQGCLPPFPADVFMIPQYGYLTLNNGSQAVGRSSFYCLEYFPSQMLRTGNNFTFSYTFEEVPFHSSYAHSQSLDRLMNPLIDQYLYYLNRTQNQSGSAQNKDLLFSRGSPAGMSVQPKNWLPGPCYRQQRVSKTKTDNNNSNFTWTGASKYNLNGRESIINPGTAMASHKDDEDKFFPMSGVMIFGKESAGASNTALDNVMITDEEEIKATNPVATERFGTVAVNFQSSSTDPATGHVHAMGALPGMVWQDRDVYLQGPIWAKIPHTDGHFHPSPLMGGFGLKNPPPQILIKNTPVPANPPAEFSATKFASFITQYSTGQVSVEIEWELQKENSKRWNPEVQYTSNYAKSANVEYTVDNNGLYTEPRPIGTRYLTRPL

SEQ ID NO: 4 - DNA, 2211 bp, synthetic construct
  source 1..2211: mol_type = other DNA
atggctgccgatggttatcttccagattggctcgaggacaacctctctgagggcattcgcgagtggtgggacttgaaacctggagccccgaagcccaaagccaaccagcaaaagcaggacgacggccggggtctggtgcttcctggctacaagtacctcggacccttcaacggactcgacaagggggagcccgtcaacgcggcggacgcagcggccctcgagcacgacaaggcctacgaccagcagctcaaagcgggtgacaatccgtaccttcggtataaccacgccgacgccgagtttcaggagcgtctgcaagaagatacgtcttttgggggcaacctcgggcgagcagtcttccaggccaagaagcgggttctcgaacctctcggtctggttgaggaaggcgctaagacggctcctggaaagaaacgtccggtagagcagtcgccacaagagccagactcctcctcgggcatcggcaagacaggccagcagcccgctaaaaagagactcaattttggtcagactggcgactcagagtcagtccccgacccacaacctctcggagaacctccagcaacccccgctgctgtgggacctactacaatggcttcaggcggtggcgcaccaatggcagacaataacgaaggcgccgacggagtgggtaatgcctcaggaaattggcattgcgattccacatggctgggcgacagagtcatcaccaccagcacccgcacctgggccttgcccacctacaataaccacctctacaagcaaatctccagtgcttcaacgggggccagcaacgacaaccactacttcggctacagcaccccctgggggtattttgatttcaacagattccactgccacttttcaccacgtgactggcagcgactcatcaacaacaattggggattccggcccaagagactcaacttcaaactcttcaacatccaagtcaaggaggtcacgacgaatgatggcgtcacaaccatcgctaataaccttaccagcacggttcaagtcttctcggactcggagtaccagcttccgtacgtcctcggctctgcgcaccagggctgcctccctccgttcccggcggacgtgttcatgattccgcaatacggctacctgacgctcaacaatggcagccaagccgtgggacgttcatccttttactgcctggaatatttcccttctcagatgctgagaacgggcaacaactttaccttcagctacacctttgaggaagtgcctttccacagcagctacgcgcacagccagagcctggaccggctgatgaatcctctcatcgaccaatacctgtattacctgaacagaactcaaaatcagtccggaagtgcccaaaacaaggacttgctgtttagccgtgggtctccagctggcatgtctgttcagcccaaaaactggctacctggaccctgttatcggcagcagcgcgtttctaaaacaaaaacagacaacaacaacagcaattttacctggactggtgcttcaaaatataacctcaatgggcgtgaatccatcatcaaccctggcactgctatggcctcacacaaagacgacgaagacaagttctttcccatgagcggtgtcatgatttttggaaaagagagcgccggagcttcaaacactgcattggacaatgtcatgattacagacgaagaggaaattaaagccactaaccctgtggccaccgaaagatttgggaccgtggcagtcaatttccagagcagcagcacagaccctgcgaccggacatgtgcatgctatgggagcattacctggcatggtgtggcaagatagagacgtgtacctgcagggtcccatttgggccaaaattcctcacacagatggacactttcacccgtctcctcttatgggcggctttggactcaagaacccgcctcctcagatcctcatcaaaaacacgcctgttcctgcgaatcctccggcggagttttcagctacaaagtttgcttcattcatcacccaatactccacaggacaagtgagtgtggaaattgaatgggagctgcagaaagaaaacagcaagcgctggaatcccgaagtgcagtacacatccaattatgcaaaatctgccaacgttgagtatactgtggacaacaatggactgtatactgagcctcgccccattggcacccgttaccttacccgtcccctgtaa

SEQ ID NO: 5 - protein, 736 aa, synthetic construct
MAADGYLPDWLEDNLSEGIREWWDLKPGAPKPKANQQKQDDGRGLVLPGYKYLGPFNGLDKGEPVNAADAAALEHDKAYDQQLKAGDNPYLRYNHADAEFQERLQEDTSFGGNLGRAVFQAKKRVLEPLGLVEEGAKTAPGKKRPVEQSPQEPDSSSGIGKTGQQPAKKRLNFGQTGDSESVPDPQPLGEPPATPAAVGPTTMASGGGAPMADNNEGADGVGNASGNWHCDSTWLGDRVITTSTRTWALPTYNNHLYKQISSASTGASNDNHYFGYSTPWGYFDFNRFHCHFSPRDWQRLINNNWGFRPKRLNFRLFNIQVKEVTTNDGVTTIANNLTSTVQVFSDSEYQLPYVLGSAHQGCLPPFPADVFMIPQYGYLTLNNGSQAVGRSSFYCLEYFPSQMLRTGNNFTFSYTFEEVPFHSSYAHSQSLDRLMNPLIDQYLYYLNRTQNQSGSAQNKDLLFSRGSPAGMSVQPKNWLPGPCYRQQRVSKTKTDNNNSNFTWTGASKYNLNGRESIINPGTAMASHKDDEDKFFPMSGVMIFGKESAGASNTALDNVMITDEEEIKATNPVATERFGTVAVNLQSSSTDPATGDVHVMGALPGMVWQDRDVYLQGPIWAKIPHTDGHFHPSPLMGGFGLKHPPPQILIKNTPVPANPPAEFSATKFASFITQYSTGQVSVEIEWELQKENSKRWNPEVQYTSNYAKSANVDFTVDNNGLYTEPRPIGTRYLTRPL

SEQ ID NO: 6 - DNA, 2211 bp, synthetic construct
  source 1..2211: mol_type = other DNA
atggctgccgatggttatcttccagattggctcgaggacaacctctctgagggcattcgcgagtggtgggacttgaaacctggagccccgaagcccaaagccaaccagcaaaagcaggacgacggccggggtctggtgcttcctggctacaagtacctcggacccttcaacggactcgacaagggggagcccgtcaacgcggcggacgcagcggccctcgagcacgacaaggcctacgaccagcagctcaaagcgggtgacaatccgtaccttcggtataaccacgccgacgccgagtttcaggagcgtctgcaagaagatacgtcttttgggggcaacctcgggcgagcagtcttccaggccaagaagcgggttctcgaacctctcggtctggttgaggaaggcgctaagacggctcctggaaagaaacgtccggtagagcagtcgccacaagagccagactcctcctcgggcatcggcaagacaggccagcagcccgctaaaaagagactcaattttggtcagactggcgactcagagtcagtccccgacccacaacctctcggagaacctccagcaacccccgctgctgtgggacctactacaatggcttcaggcggtggcgcaccaatggcagacaataacgaaggcgccgacggagtgggtaatgcctcaggaaattggcattgcgattccacatggctgggcgacagagtcatcaccaccagcacccgcacctgggccttgcccacctacaataaccacctctacaagcaaatctccagtgcttcaacgggggccagcaacgacaaccactacttcggctacagcaccccctgggggtattttgatttcaacagattccactgccacttttcaccacgtgactggcagcgactcatcaacaacaattggggattccggcccaagagactcaacttcagactcttcaacatccaagtcaaggaggtcacgacgaatgatggcgtcacaaccatcgctaataaccttaccagcacggttcaagtcttctcggactcggagtaccagcttccgtacgtcctcggctctgcgcaccagggctgcctccctccgttcccggcggacgtgttcatgattccgcaatacggctacctgacgctcaacaatggcagccaagccgtgggacgttcatccttttactgcctggaatatttcccttctcagatgctgagaacgggcaacaactttaccttcagctacacctttgaggaagtgcctttccacagcagctacgcgcacagccagagcctggaccggctgatgaatcctctcatcgaccaatacctgtattacctgaacagaactcaaaatcagtccggaagtgcccaaaacaaggacttgctgtttagccgtgggtctccagctggcatgtctgttcagcccaaaaactggctacctggaccctgttatcggcagcagcgcgtttctaaaacaaaaacagacaacaacaacagcaattttacctggactggtgcttcaaaatataacctcaatgggcgtgaatccatcatcaaccctggcactgctatggcctcacacaaagacgacgaagacaagttctttcccatgagcggtgtcatgatttttggaaaagagagcgccggagcttcaaacactgcattggacaatgtcatgattacagacgaagaggaaatcaaagccactaaccccgtggccaccgaaagatttgggactgtggcagtcaatctccagagcagcagcacagaccctgcgaccggagatgtgcatgttatgggagccttacctggaatggtgtggcaagacagagacgtatacctgcagggtcctatttgggccaaaattcctcacacggatggacactttcacccgtctcctctcatgggcggctttggacttaagcacccgcctcctcagatcctcatcaaaaacacgcctgttcctgcgaatcctccggcagagttttcggctacaaagtttgcttcattcatcacccagtattccacaggacaagtgagcgtggagattgaatgggagctgcagaaagaaaacagcaaacgctggaatcccgaagtgcagtatacatctaactatgcaaaatctgccaacgttgatttcactgtggacaacaatggactttatactgagcctcgccccattggcacccgttacctcacccgtcccctgtaa

SEQ ID NO: 7 - DNA, 8343 bp, synthetic construct
  source 1..8343: mol_type = other DNA
ctggcgtaatagcgaagaggcccgcaccgatcgcccttcccaacagttgcgcagcctgaatggcgaatggcgattccgttgcaatggctggcggtaatattgttctggatattaccagcaaggccgatagtttgagttcttctactcaggcaagtgatgttattactaatcaaagaagtattgcgacaacggttaatttgcgtgatggacagactcttttactcggtggcctcactgattataaaaacacttctcaggattctggcgtaccgttcctgtctaaaatccctttaatcggcctcctgtttagctcccgctctgattctaacgaggaaagcacgttatacgtgctcgtcaaagcaaccatagtacgcgccctgtagcggcgcattaagcgcggcgggtgtggtggttacgcgcagcgtgaccgctacacttgccagcgccctagcgcccgctcctttcgctttcttcccttcctttctcgccacgttcgccggctttccccgtcaagctctaaatcgggggctccctttagggttccgatttagtgctttacggcacctcgaccccaaaaaacttgattagggtgatggttcacgtagtgggccatcgccctgatagacggtttttcgccctttgacgttggagtccacgttctttaatagtggactcttgttccaaactggaacaacactcaaccctatctcggtctattcttttgatttataagggattttgccgatttcggcatattggttaaaaaatgagctgatttaacaaaaatttaacgcgaattttaacaaaatattaacgcttacaatttaaatatttgcttatacaatcttcctgtttttggggcttttctgattatcaaccggggtacatatgattgacatgctagttttacgattaccgttcatcgattctcttgtttgctccagactctcaggcaatgacctgatagcctttgtagagacctctcaaaaatagctaccctctccggcatgaatttatcagctagaacggttgaatatcatattgatggtgatttgactgtctccggcctttctcacccgtttgaatctttacctacacattactcaggcattgcatttaaaatatatgagggttctaaaaatttttatccttgcgttgaaataaaggcttctcccgcaaaagtattacagggtcataatgtttttggtacaaccgatttagctttatgctctgaggctttattgcttaattttgctaattctttgccttgcctgtatgatttattggatgttggaatcgcctgatgcggtattttctccttacgcatctgtgcggtatttcacaccgcatatggtgcactctcagtacaatctgctctgatgccgcatagttaagccagccccgacacccgccaacacccgctgacgcgccctgacgggcttgtctgctcccggcatccgcttacagacaagctgtgaccgtctccgggagctgcatgtgtcagaggttttcaccgtcatcaccgaaacgcgcgagacgaaagggcctcgtgatacgcctatttttataggttaatgtcatgataataatggtttcttagacgtcaggtggcacttttcggggaaatgtgcgcggaacccctatttgtttatttttctaaatacattcaaatatgtatccgctcatgagacaataaccctgataaatgcttcaataatattgaaaaaggaagagtatgagtattcaacatttccgtgtcgcccttattcccttttttgcggcattttgccttcctgtttttgctcacccagaaacgctggtgaaagtaaaagatgctgaagatcagttgggtgcacgagtgggttacatcgaactggatctcaacagcggtaagatccttgagagttttcgccccgaagaacgttttccaatgatgagcacttttaaagttctgctatgtggcgcggtattatcccgtattgacgccgggcaagagcaactcggtcgccgcatacactattctcagaatgacttggttgagtactcaccagtcacagaaaagcatcttacggatggcatgacagtaagagaattatgcagtgctgccataaccatgagtgataacactgcggccaacttacttctgacaacgatcggaggaccgaaggagctaaccgcttttttgcacaacatgggggatcatgtaactcgccttgatcgttgggaaccggagctgaatgaagccataccaaacgacgagcgtgacaccacgatgcctgtagcaatggcaacaacgttgcgcaaactattaactggcgaactacttactctagcttcccggcaacaattaatagactggatggaggcggataaagttgcaggaccacttctgcgctcggcccttccggctggctggtttattgctgataaatctggagccggtgagcgtgggtctcgcggtatcattgcagcactggggccagatggtaagccctcccgtatcgtagttatctacacgacggggagtcaggcaactatggatgaacgaaatagacagatcgctgagataggtgcctcactgattaagcattggtaactgtcagaccaagtttactcatatatactttagattgatttaaaacttcatttttaatttaaaaggatctaggtgaagatcctttttgataatctcatgaccaaaatcccttaacgtgagttttcgttccactgagcgtcagaccccgtagaaaagatcaaaggatcttcttgagatcctttttttctgcgcgtaatctgctgcttgcaaacaaaaaaaccaccgctaccagcggtggtttgtttgccggatcaagagctaccaactctttttccgaaggtaactggcttcagcagagcgcagataccaaatactgttcttctagtgtagccgtagttaggccaccacttcaagaactctgtagcaccgcctacatacctcgctctgctaatcctgttaccagtggctgctgccagtggcgataagtcgtgtcttaccgggttggactcaagacgatagttaccggataaggcgcagcggtcgggctgaacggggggttcgtgcacacagcccagcttggagcgaacgacctacaccgaactgagatacctacagcgtgagctatgagaaagcgccacgcttcccgaagggagaaaggcggacaggtatccggtaagcggcagggtcggaacaggagagcgcacgagggagcttccagggggaaacgcctggtatctttatagtcctgtcgggtttcgccacctctgacttgagcgtcgatttttgtgatgctcgtcaggggggcggagcctatggaaaaacgccagcaacgcggcctttttacggttcctggccttttgctggccttttgctcaccatgttctttcctgcgttatcccctgattctgtggataaccgtattacccgctttgagtgagctgataccgctcgccgcagccgaacgaccgagcgcagcgagtcagtgagcgaggaagcggaagagcgcccaatacgcaaaccgcctctccccgcgcgttggccgattcattaatgcagaattcccatcatcaataatataccttattttggattgaagccaatatgataatgagggggtggagtttgtgacgtggcgcggggcgtgggaacggggcgggtgacgtagtagctctagaggtcctgtattagaggtcacgtgagtgttttgcgacattttgcgacaccatgtggtcacgctgggtatttaagcccgagtgagcacgcagggtctccattttgaagcgggaggtttgaacgcgcagccaccacggcggggttttacgagattgtgattaaggtccccagcgaccttgacgagcatctgcccggcatttctgacagctttgtgaactgggtggccgagaaggaatgggagttgccgccagattctgacatggatctgaatctgattgagcaggcacccctgaccgtggccgagaagctgcagcgcgactttctgacggaatggcgccgtgtgagtaaggccccggaggcccttttctttgtgcaatttgagaagggagagagctacttccacatgcacgtgctcgtggaaaccaccggggtgaaatccatggttttgggacgtttcctgagtcagattcgcgaaaaactgattcagagaatttaccgcgggatcgagccgactttgccaaactggttcgcggtcacaaagaccagaaatggcgccggaggcgggaacaaggtggtggatgagtgctacatccccaattacttgctccccaaaacccagcctgagctccagtgggcgtggactaatatggaacagtatttaagcgcctgtttgaatctcacggagcgtaaacggttggtggcgcagcatctgacgcacgtgtcgcagacgcaggagcagaacaaagagaatcagaatcccaattctgatgcgccggtgatcagatcaaaaacttcagccaggtacatggagctggtcgggtggctcgtggacaaggggattacctcggagaagcagtggatccaggaggaccaggcctcatacatctccttcaatgcggcctccaactcgcggtcccaaatcaaggctgccttggacaatgcgggaaagattatgagcctgactaaaaccgcccccgactacctggtgggccagcagcccgtggaggacatttccagcaatcggatttataaaattttggaactaaacgggtacgatccccaatatgcggcttccgtctttctgggatgggccacgaaaaagttcggcaagaggaacaccatctggctgtttgggcctgcaactaccgggaagaccaacatcgcggaggccatagcccacactgtgcccttctacgggtgcgtaaactggaccaatgagaactttcccttcaacgactgtgtcgacaagatggtgatctggtgggaggaggggaagatgaccgccaaggtcgtggagtcggccaaagccattctcggaggaagcaaggtgcgcgtggaccagaaatgcaagtcctcggcccagatagacccgactcccgtgatcgtcacctccaacaccaacatgtgcgccgtgattgacgggaactcaacgaccttcgaacaccagcagccgttgcaagaccggatgttcaaatttgaactcacccgccgtctggatcatgactttgggaaggtcaccaagcaggaagtcaaagactttttccggtgggcaaaggatcacgtggttgaggtggagcatgaattctacgtcaaaaagggtggagccaagaaaagacccgcccccagtgacgcagatataagtgagcccaaacgggtgcgcgagtcagttgcgcagccatcgacgtcagacgcggaagcttcgatcaactacgcagacaggtaccaaaacaaatgttctcgtcacgtgggcatgaatctgatgctgtttccctgcagacaatgcgagagaatgaatcagaattcaaatatctgcttcactcacggacagaaagactgtttagagtgctttcccgtgtcagaatctcaacccgtttctgtcgtcaaaaaggcgtatcagaaactgtgctacattcatcatatcatgggaaaggtgccagacgcttgcactgcctgcgatctggtcaatgtggatttggatgactgcatctttgaacaataaatgatttaaatcaggtatggctgccgatggttatcttccagattggctcgaggacaacctctctgagggcattcgcgagtggtgggacttgaaacctggagccccgaagcccaaagccaaccagcaaaagcaggacgacggccggggtctggtgcttcctggctacaagtacctcggacccttcaacggactcgacaagggggagcccgtcaacgcggcggacgcagcggccctcgagcacgacaaggcctacgaccagcagctcaaagcgggtgacaatccgtaccttcggtataaccacgccgacgccgagtttcaggagcgtctgcaagaagatacgtcttttgggggcaacctcgggcgagcagtcttccaggccaagaagcgggttctcgaacctctcggtctggttgaggaaggcgctaagacggctcctggaaagaaacgtccggtagagcagtcgccacaagagccagactcctcctcgggcatcggcaagacaggccagcagcccgctaaaaagagactcaattttggtcagactggcgactcagagtcagtccccgacccacaacctctcggagaacctccagcaacccccgctgctgtgggacctactacaatggcttcaggcggtggcgcaccaatggcagacaataacgaaggcgccgacggagtgggtaatgcctcaggaaattggcattgcgattccacatggctgggcgacagagtcatcaccaccagcacccgcacctgggccttgcccacctacaataaccacctctacaagcaaatctccagtgcttcaacgggggccagcaacgacaaccactacttcggctacagcaccccctgggggtattttgatttcaacagattccactgccacttttcaccacgtgactggcagcgactcatcaacaacaattggggattccggcccaagagactcaacttcaaactcttcaacatccaagtcaaggaggtcacgacgaatgatggcgtcacaaccatcgctaataaccttaccagcacggttcaagtcttctcggactcggagtaccagcttccgtacgtcctcggctctgcgcaccagggctgcctccctccgttcccggcggacgtgttcatgattccgcaatacggctacctgacgctcaacaatggcagccaagccgtgggacgttcatccttttactgcctggaatatttcccttctcagatgctgagaacgggcaacaactttaccttcagctacacctttgaggaagtgcctttccacagcagctacgcgcacagccagagcctggaccggctgatgaatcctctcatcgaccaatacctgtattacctgaacagaactcaaaatcagtccggaagtgcccaaaacaaggacttgctgtttagccgtgggtctccagctggcatgtctgttcagcccaaaaactggctacctggaccctgttatcggcagcagcgcgtttctaaaacaaaaacagacaacaacaacagcaattttacctggactggtgcttcaaaatataacctcaatgggcgtgaatccatcatcaaccctggcactgctatggcctcacacaaagacgacgaagacaagttctttcccatgagcggtgtcatgatttttggaaaagagagcgccggagcttcaaacactgcattggacaatgtcatgattacagacgaagaggaaattaaagccactaaccctgtggccaccgaaagatttgggaccgtggcagtcaatttccagagcagcagcacagaccctgcgaccggacatgtgcatgctatgggagcattacctggcatggtgtggcaagatagagacgtgtacctgcagggtcccatttgggccaaaattcctcacacagatggacactttcacccgtctcctcttatgggcggctttggactcaagaacccgcctcctcagatcctcatcaaaaacacgcctgttcctgcgaatcctccggcggagttttcagctacaaagtttgcttcattcatcacccaatactccacaggacaagtgagtgtggaaattgaatgggagctgcagaaagaaaacagcaagcgctggaatcccgaagtgcagtacacatccaattatgcaaaatctgccaacgttgagtatactgtggacaacaatggactgtatactgagcctcgccccattggcacccgttaccttacccgtcccctgtaattgcggccgcttgttaatcaataaaccgtttaattcgtttcagttgaactttggtctctgcgtatttctttcttatctagtttccatgctctagaggtcctgtattagaggtcacgtgagtgttttgcgacattttgcgacaccatgtggtcacgctgggtatttaagcccgagtgagcacgcagggtctccattttgaagcgggaggtttgaacgcgcagccaccacggcggggttttacgagattgtgattaaggtccccagcgaccttgacgagcatctgcccggcatttctgacagctttgtgaactgggtggccgagaaggaatgggagttgccgccagattctgacatggatctgaatctgattgagcaggcacccctgaccgtggccgagaagctgcatcg

SEQ ID NO: 8 - DNA, 8343 bp, synthetic construct
  source 1..8343: mol_type = other DNA
ctggcgtaatagcgaagaggcccgcaccgatcgcccttcccaacagttgcgcagcctgaatggcgaatggcgattccgttgcaatggctggcggtaatattgttctggatattaccagcaaggccgatagtttgagttcttctactcaggcaagtgatgttattactaatcaaagaagtattgcgacaacggttaatttgcgtgatggacagactcttttactcggtggcctcactgattataaaaacacttctcaggattctggcgtaccgttcctgtctaaaatccctttaatcggcctcctgtttagctcccgctctgattctaacgaggaaagcacgttatacgtgctcgtcaaagcaaccatagtacgcgccctgtagcggcgcattaagcgcggcgggtgtggtggttacgcgcagcgtgaccgctacacttgccagcgccctagcgcccgctcctttcgctttcttcccttcctttctcgccacgttcgccggctttccccgtcaagctctaaatcgggggctccctttagggttccgatttagtgctttacggcacctcgaccccaaaaaacttgattagggtgatggttcacgtagtgggccatcgccctgatagacggtttttcgccctttgacgttggagtccacgttctttaatagtggactcttgttccaaactggaacaacactcaaccctatctcggtctattcttttgatttataagggattttgccgatttcggcatattggttaaaaaatgagctgatttaacaaaaatttaacgcgaattttaacaaaatattaacgcttacaatttaaatatttgcttatacaatcttcctgtttttggggcttttctgattatcaaccggggtacatatgattgacatgctagttttacgattaccgttcatcgattctcttgtttgctccagactctcaggcaatgacctgatagcctttgtagagacctctcaaaaatagctaccctctccggcatgaatttatcagctagaacggttgaatatcatattgatggtgatttgactgtctccggcctttctcacccgtttgaatctttacctacacattactcaggcattgcatttaaaatatatgagggttctaaaaatttttatccttgcgttgaaataaaggcttctcccgcaaaagtattacagggtcataatgtttttggtacaaccgatttagctttatgctctgaggctttattgcttaattttgctaattctttgccttgcctgtatgatttattggatgttggaatcgcctgatgcggtattttctccttacgcatctgtgcggtatttcacaccgcatatggtgcactctcagtacaatctgctctgatgccgcatagttaagccagccccgacacccgccaacacccgctgacgcgccctgacgggcttgtctgctcccggcatccgcttacagacaagctgtgaccgtctccgggagctgcatgtgtcagaggttttcaccgtcatcaccgaaacgcgcgagacgaaagggcctcgtgatacgcctatttttataggttaatgtcatgataataatggtttcttagacgtcaggtggcacttttcggggaaatgtgcgcggaacccctatttgtttatttttctaaatacattcaaatatgtatccgctcatgagacaataaccctgataaatgcttcaataatattgaaaaaggaagagtatgagtattcaacatttccgtgtcgcccttattcccttttttgcggcattttgccttcctgtttttgctcacccagaaacgctggtgaaagtaaaagatgctgaagatcagttgggtgcacgagtgggttacatcgaactggatctcaacagcggtaagatccttgagagttttcgccccgaagaacgttttccaatgatgagcacttttaaagttctgctatgtggcgcggtattatcccgtattgacgccgggcaagagcaactcggtcgccgcatacactattctcagaatgacttggttgagtactcaccagtcacagaaaagcatcttacggatggcatgacagtaagagaattatgcagtgctgccataaccatgagtgataacactgcggccaacttacttctgacaacgatcggaggaccgaaggagctaaccgcttttttgcacaacatgggggatcatgtaactcgccttgatcgttgggaaccggagctgaatgaagccataccaaacgacgagcgtgacaccacgatgcctgtagcaatggcaacaacgttgcgcaaactattaactggcgaactacttactctagcttcccggcaacaattaatagactggatggaggcggataaagttgcaggaccacttctgcgctcggcccttccggctggctggtttattgctgataaatctggagccggtgagcgtgggtctcgcggtatcattgcagcactggggccagatggtaagccctcccgtatcgtagttatctacacgacggggagtcaggcaactatggatgaacgaaatagacagatcgctgagataggtgcctcactgattaagcattggtaactgtcagaccaagtttactcatatatactttagattgatttaaaacttcatttttaatttaaaaggatctaggtgaagatcctttttgataatctcatgaccaaaatcccttaacgtgagttttcgttccactgagcgtcagaccccgtagaaaagatcaaaggatcttcttgagatcctttttttctgcgcgtaatctgctgcttgcaaacaaaaaaaccaccgctaccagcggtggtttgtttgccggatcaagagctaccaactctttttccgaaggtaactggcttcagcagagcgcagataccaaatactgttcttctagtgtagccgtagttaggccaccacttcaagaactctgtagcaccgcctacatacctcgctctgctaatcctgttaccagtggctgctgccagtggcgataagtcgtgtcttaccgggttggactcaagacgatagttaccggataaggcgcagcggtcgggctgaacggggggttcgtgcacacagcccagcttggagcgaacgacctacaccgaactgagatacctacagcgtgagctatgagaaagcgccacgcttcccgaagggagaaaggcggacaggtatccggtaagcggcagggtcggaacaggagagcgcacgagggagcttccagggggaaacgcctggtatctttatagtcctgtcgggtttcgccacctctgacttgagcgtcgatttttgtgatgctcgtcaggggggcggagcctatggaaaaacgccagcaacgcggcctttttacggttcctggccttttgctggccttttgctcaccatgttctttcctgcgttatcccctgattctgtggataaccgtattacccgctttgagtgagctgataccgctcgccgcagccgaacgaccgagcgcagcgagtcagtgagcgaggaagcggaagagcgcccaatacgcaaaccgcctctccccgcgcgttggccgattcattaatgcagaattcccatcatcaataatataccttattttggattgaagccaatatgataatgagggggtggagtttgtgacgtggcgcggggcgtgggaacggggcgggtgacgtagtagctctagaggtcctgtattagaggtcacgtgagtgttttgcgacattttgcgacaccatgtggtcacgctgggtatttaagcccgagtgagcacgcagggtctccattttgaagcgggaggtttgaacgcgcagccaccacggcggggttttacgagattgtgattaaggtccccagcgaccttgacgagcatctgcccggcatttctgacagctttgtgaactgggtggccgagaaggaatgggagttgccgccagattctgacatggatctgaatctgattgagcaggcacccctgaccgtggccgagaagctgcagcgcgactttctgacggaatggcgccgtgtgagtaaggccccggaggcccttttctttgtgcaatttgagaagggagagagctacttccacatgcacgtgctcgtggaaaccaccggggtgaaatccatggttttgggacgtttcctgagtcagattcgcgaaaaactgattcagagaatttaccgcgggatcgagccgactttgccaaactggttcgcggtcacaaagaccagaaatggcgccggaggcgggaacaaggtggtggatgagtgctacatccccaattacttgctccccaaaacccagcctgagctccagtgggcgtggactaatatggaacagtatttaagcgcctgtttgaatctcacggagcgtaaacggttggtggcgcagcatctgacgcacgtgtcgcagacgcaggagcagaacaaagagaatcagaatcccaattctgatgcgccggtgatcagatcaaaaacttcagccaggtacatggagctggtcgggtggctcgtggacaaggggattacctcggagaagcagtggatccaggaggaccaggcctcatacatctccttcaatgcggcctccaactcgcggtcccaaatcaaggctgccttggacaatgcgggaaagattatgagcctgactaaaaccgcccccgactacctggtgggccagcagcccgtggaggacatttccagcaatcggatttataaaattttggaactaaacgggtacgatccccaatatgcggcttccgtctttctgggatgggccacgaaaaagttcggcaagaggaacaccatctggctgtttgggcctgcaactaccgggaagaccaacatcgcggaggccatagcccacactgtgcccttctacgggtgcgtaaactggaccaatgagaactttcccttcaacgactgtgtcgacaagatggtgatctggtgggaggaggggaagatgaccgccaaggtcgtggagtcggccaaagccattctcggaggaagcaaggtgcgcgtggaccagaaatgcaagtcctcggcccagatagacccgactcccgtgatcgtcacctccaacaccaacatgtgcgccgtgattgacgggaactcaacgaccttcgaacaccagcagccgttgcaagaccggatgttcaaatttgaactcacccgccgtctggatcatgactttgggaaggtcaccaagcaggaagtcaaagactttttccggtgggcaaaggatcacgtggttgaggtggagcatgaattctacgtcaaaaagggtggagccaagaaaagacccgcccccagtgacgcagatataagtgagcccaaacgggtgcgcgagtcagttgcgcagccatcgacgtcagacgcggaagcttcgatcaactacgcagacaggtaccaaaacaaatgttctcgtcacgtgggcatgaatctgatgctgtttccctgcagacaatgcgagagaatgaatcagaattcaaatatctgcttcactcacggacagaaagactgtttagagtgctttcccgtgtcagaatctcaacccgtttctgtcgtcaaaaaggcgtatcagaaactgtgctacattcatcatatcatgggaaaggtgccagacgcttgcactgcctgcgatctggtcaatgtggatttggatgactgcatctttgaacaataaatgatttaaatcaggtatggctgccgatggttatcttccagattggctcgaggacaacctctctgagggcattcgcgagtggtgggacttgaaacctggagccccgaagcccaaagccaaccagcaaaagcaggacgacggccggggtctggtgcttcctggctacaagtacctcggacccttcaacggactcgacaagggggagcccgtcaacgcggcggacgcagcggccctcgagcacgacaaggcctacgaccagcagctcaaagcgggtgacaatccgtaccttcggtataaccacgccgacgccgagtttcaggagcgtctgcaagaagatacgtcttttgggggcaacctcgggcgagcagtcttccaggccaagaagcgggttctcgaacctctcggtctggttgaggaaggcgctaagacggctcctggaaagaaacgtccggtagagcagtcgccacaagagccagactcctcctcgggcatcggcaagacaggccagcagcccgctaaaaagagactcaattttggtcagactggcgactcagagtcagtccccgacccacaacctctcggagaacctccagcaacccccgctgctgtgggacctactacaatggcttcaggcggtggcgcaccaatggcagacaataacgaaggcgccgacggagtgggtaatgcctcaggaaattggcattgcgattccacatggctgggcgacagagtcatcaccaccagcacccgcacctgggccttgcccacctacaataaccacctctacaagcaaatctccagtgcttcaacgggggccagcaacgacaaccactacttcggctacagcaccccctgggggtattttgatttcaacagattccactgccacttttcaccacgtgactggcagcgactcatcaacaacaattggggattccggcccaagagactcaacttcagactcttcaacatccaagtcaaggaggtcacgacgaatgatggcgtcacaaccatcgctaataaccttaccagcacggttcaagtcttctcggactcggagtaccagcttccgtacgtcctcggctctgcgcaccagggctgcctccctccgttcccggcggacgtgttcatgattccgcaatacggctacctgacgctcaacaatggcagccaagccgtgggacgttcatccttttactgcctggaatatttcccttctcagatgctgagaacgggcaacaactttaccttcagctacacctttgaggaagtgcctttccacagcagctacgcgcacagccagagcctggaccggctgatgaatcctctcatcgaccaatacctgtattacctgaacagaactcaaaatcagtccggaagtgcccaaaacaaggacttgctgtttagccgtgggtctccagctggcatgtctgttcagcccaaaaactggctacctggaccctgttatcggcagcagcgcgtttctaaaacaaaaacagacaacaacaacagcaattttacctggactggtgcttcaaaatataacctcaatgggcgtgaatccatcatcaaccctggcactgctatggcctcacacaaagacgacgaagacaagttctttcccatgagcggtgtcatgatttttggaaaagagagcgccggagcttcaaacactgcattggacaatgtcatgattacagacgaagaggaaatcaaagccactaaccccgtggccaccgaaagatttgggactgtggcagtcaatctccagagcagcagcacagaccctgcgaccggagatgtgcatgttatgggagccttacctggaatggtgtggcaagacagagacgtatacctgcagggtcctatttgggccaaaattcctcacacggatggacactttcacccgtctcctctcatgggcggctttggacttaagcacccgcctcctcagatcctcatcaaaaacacgcctgttcctgcgaatcctccggcagagttttcggctacaaagtttgcttcattcatcacccagtattccacaggacaagtgagcgtggagattgaatgggagctgcagaaagaaaacagcaaacgctggaatcccgaagtgcagtatacatctaactatgcaaaatctgccaacgttgatttcactgtggacaacaatggactttatactgagcctcgccccattggcacccgttacctcacccgtcccctgtaattgcggccgcttgttaatcaataaaccgtttaattcgtttcagttgaactttggtctctgcgtatttctttcttatctagtttccatgctctagaggtcctgtattagaggtcacgtgagtgttttgcgacattttgcgacaccatgtggtcacgctgggtatttaagcccgagtgagcacgcagggtctccattttgaagcgggaggtttgaacgcgcagccaccacggcggggttttacgagattgtgattaaggtccccagcgaccttgacgagcatctgcccggcatttctgacagctttgtgaactgggtggccgagaaggaatgggagttgccgccagattctgacatggatctgaatctgattgagcaggcacccctgaccgtggccgagaagctgcatcg

SEQ ID NO: 9 - DNA, 23 bp, synthetic construct
  source 1..23: mol_type = other DNA
gcggaagcttcgatcaactacgc

SEQ ID NO: 10 - DNA, 40 bp, synthetic construct
  source 1..40: mol_type = other DNA
gggcggccgcaattacagattacgagtcaggtatctggtg

SEQ ID NO: 11 - protein, 19 aa, synthetic construct
ATNFSLLKQAGDVEENPGP